European Patent Application EP 4 649 949 A1, published November 19, 2025. Title: Pharmaceutical composition for preventing proliferative vitreoretinopathy comprising autotaxin aptamer. Applicant: RIBOMIC INC. The sequence listing filed with the application follows.

SEQUENCE LISTING (3 sequences)

SEQ ID NO: 1 - RNA, 15 nt, synthetic construct
  source 1..15: mol_type = other RNA
gwaacaggttttgct

SEQ ID NO: 2 - RNA, 29 nt, synthetic construct
  source 1..29: mol_type = other RNA
tctgagggaaacaggttttgctcctcgga

SEQ ID NO: 3 - RNA, 15 nt, synthetic construct
  source 1..15: mol_type = other RNA
gaaacaggttttgct